European Patent Specification EP 4 074 817 B1, published April 8, 2026. Title: Lactobacillus Rhamnosus X253 Beneficial to Oral Health, Separation and Purification Method and Use Thereof. Applicant: THE SHIJIAZHUANG JUNLEBAO DAIRY CO., LTD. The sequence listing filed with the application follows.

SEQUENCE LISTING (2 sequences)

SEQ ID NO: 1 - DNA, 1451 bp, Lactobacillus rhamnosus
cttagacggctcgctccctaaaagggttacgccaccggcttcgggtgttacaaactctcatggtgtgacgggcggtgtgtacaaggcccgggaacgtattcaccgcggcgtgctgatccgcgattactagcgattccgacttcgtgtaggcgagttgcagcctacagtccgaactgagaatggctttaagagattagcttgacctcgcggtctcgcaacctcgttgtacccatccattgtagcacgtgtgtagcccaggtcataaggggcatgatgatttgacgtcatccccaccttcctccggtttgtcaccggcaggtcttactagagtgcccaactaaatgctggcaactagtcataagggttgcgctcgttgcgggacttaacccaacatctcacgacacgagctgacgacaaccatgcaccacctgtcattttgcccccgaaggggaaacctgatctctcaggtgatcaaaagatgtcaagacctggtaaggttcttcgcgttgcttcgaattaaaccacatgctccaccgcttgtgcgggcccccgtcaattcctttgagtttcaaccttgcggtcgtactcccaggcggaatgcttaatgcgttagctgcggcactgaagggcggaaaccctccaacacctagcattcatcgtttacggcattggactaccagggtatctaatcctgttcgctacccatgctttcgagcctcagcgtcagttacagaccagacagccgccttcgccactggtgttcttccatatatctacgcatttcaccagctacacatggagttccactgtcctcttctgcactcaagtttcccagtttccgatgcacttcctcggttaagccgagggctttcacatcagacttaaaaaaccgcctgcgctcgctttacgcccaataaatccggataacgcttgccacctacgtattaccgcggctgctggcacgtagttagccgtggctttctggttggataccgtcacgccgacaacagttactctgccgaccattcttctccacaacagagttttacgacccgaaagccttcttcactcacgcggcgttgctccatcagacttgcgtccattgtggaagattccctactgctgcctcccgtaggagtttgggccgtgtctcagtcccaaatgtggccgatcaacctctcagttcggctacgtatcattgccttggtgagccgttacctcaccaactagctaatacgccgcgggtccatccaaaagcgatagcttacgccatctttcagccaagaaccatgcggttcttggatttatgcggtattagcatctgtttccaaatgttatcccccacttaagggcaggttacccacgtgttactcacccgtcgccactcgttcaaaattaaatcaagatgcaagcacctttcaataatcagaactcgttcgacttgcatgtat

SEQ ID NO: 2 - DNA, 468 bp, Lactobacillus rhamnosus
gggggaaaaatagccgcacgcaaacattcggatgcaccatgccggcaccgagaacttcaatccagccggtatacttgcaaacagggcaacccttgccaccgcagcggaagcaggaaacgtccacttctacagacggttctgtaaacggaaaatagctcgggcgcaggcgaatcgtccgatcagcgccaaacacatgctgacacatggcgagtaacgtccccttaagatcagccattgtaatatgcttgtcgatcaccagaccttccatctgatggaactggtggctatgtgtggcatcatcatcatcacgccgataaaccacgcccggactgatcattttcagcgggcccttagtaaaatcatgtttctccatcgtccgtgcctgcatcgggctggtttgggaacgcatcagcaactcattggtaatataaaaagtttcctgcatatcacgagcatggatgacgccga